European Patent Specification EP 3 684 794 B1, published August 6, 2025. Title: SOMATOSTATIN PRODRUGS. Applicant: YISSUM RESEARCH DEVELOPMENT COMPANY OF THE HEBREW UNIVERSITY OF JERUSALEM LTD. The sequence listing filed with the application follows.

SEQUENCE LISTING (23 sequences)

SEQ ID NO: 1 - protein, 8 aa, Artificial Sequence
  Synthetic peptide
  MISC_FEATURE (1)..(1): D-Phe
  DISULFID (2)..(7): bridge
  MISC_FEATURE (4)..(4): D-Trp
  MISC_FEATURE (8)..(8): (ol) = alcohol C termuinus
FCFWKTCT

SEQ ID NO: 2 - protein, 8 aa, Artificial Sequence
  Synthetic peptide
  MOD_RES (1)..(1): X = D-2 naphthylalanine
  DISULFID (2)..(7): bridge
  MOD_RES (4)..(4): D-Trp
  MOD_RES (8)..(8): AMIDATION
XCYWKVCT

SEQ ID NO: 3 - protein, 8 aa, Artificial Sequence
  Synthetic peptide
  MOD_RES (1)..(1): 4Abu, GABA
  MOD_RES (1)..(8): backbone-to-end cyclization between the N-alpha-omega-functionalized derivative of GlyC3 and the N-terminus
  MOD_RES (4)..(4): D-Trp
  MOD_RES (8)..(8): AMIDATION
  MOD_RES (8)..(8): GlyC3 building unit
XFWWKTFG

SEQ ID NO: 4 - protein, 6 aa, Artificial Sequence
  Synthetic peptide
  MOD_RES (1)..(1): (2-aminoethyl-carbamoyl)-Hydroxyproline
  MOD_RES (1)..(6): head-to-tail cyclization
  MOD_RES (2)..(2): PhenylGlycine, Phg
  MOD_RES (3)..(3): D-Trp
  MOD_RES (5)..(5): Tyr(Bzl)
XXWKYF

SEQ ID NO: 5 - protein, 4 aa, Artificial Sequence
  Synthetic peptide
FWKT

SEQ ID NO: 6 - protein, 4 aa, Artificial Sequence
  Synthetic peptide
  MOD_RES (2)..(2): D-Trp
FWKT

SEQ ID NO: 7 - protein, 6 aa, Artificial Sequence
  Synthetic peptide
  MOD_RES (1)..(6): head-to-tail-cyclization
  MOD_RES (3)..(3): D-Trp
PFWKTF

SEQ ID NO: 8 - protein, 6 aa, Artificial Sequence
  Synthetic peptide
  MOD_RES (1)..(6): head-to-tail cyclization
  MOD_RES (3)..(3): N-methyl D-Trp
  MOD_RES (4)..(4): N-methyl Lys
  MOD_RES (6)..(6): N-methyl Phe
PFWKTF

SEQ ID NO: 9 - protein, 7 aa, Artificial Sequence
  Synthetic peptide
  MOD_RES (1)..(1): PheN2 building unit
  MOD_RES (1)..(6): backbone cyclization between the N-alpha-omega-functionalized derivative of X1 and the N-alpha-omega-functionalized derivative of X6
  MOD_RES (3)..(3): D-Trp
  MOD_RES (6)..(6): PheC3 building unit
  MOD_RES (7)..(7): AMIDATION
FYWKVFT

SEQ ID NO: 10 - protein, 9 aa, Artificial Sequence
  Synthetic peptide
  MOD_RES (1)..(1): PheC3 building unit
  MOD_RES (1)..(9): backbone cyclization between the N-alpha-omega-functionalized derivative of X1 and the N-alpha-omega-functionalized derivative of X9
  DISULFID (2)..(7): bridge
  MOD_RES (4)..(4): D-Trp
  MOD_RES (9)..(9): PheN3 building unit
  MOD_RES (9)..(9): AMIDATION
FCFWKTCFF

SEQ ID NO: 11 - protein, 4 aa, Artificial Sequence
  Synthetic peptide
  MOD_RES (1)..(1): N-METHYL D-Trp
  MOD_RES (2)..(2): N-METHYL Lys
  MOD_RES (4)..(4): N-METHYL Phe
WKTF

SEQ ID NO: 12 - protein, 6 aa, Artificial Sequence
  Synthetic peptide
  MOD_RES (1)..(6): head-to-tail cyclization
  MOD_RES (3)..(3): N-methyl D-Trp
  MOD_RES (4)..(4): N-methyl Lys
  MOD_RES (6)..(6): N-methyl Phe
FWWKTF

SEQ ID NO: 13 - protein, 6 aa, Artificial Sequence
  Synthetic peptide
  MOD_RES (1)..(6): Backbone-to-end cyclization between the N-alpha-omega-functionalized derivative of X6 and the N terminus
  MOD_RES (4)..(4): D-Trp
  MOD_RES (5)..(5): D-Lys
  MOD_RES (6)..(6): AMIDATION
  MOD_RES (6)..(6): PheC2 building unit
FFFWKF

SEQ ID NO: 14 - protein, 6 aa, Artificial Sequence
  Synthetic peptide
  MOD_RES (1)..(1): PheC1 building unit
  MOD_RES (1)..(6): backbone cyclization between the N-alpha-omega-functionalized derivative of X1 and the N-alpha-omega-functionalized derivative of X6
  MOD_RES (4)..(4): D-Trp
  MOD_RES (6)..(6): AMIDATION
  MOD_RES (6)..(6): PheN2 building unit
FFFWKF

SEQ ID NO: 15 - protein, 6 aa, Artificial Sequence
  Synthetic peptide
  MOD_RES (1)..(1): PheC1 building unit
  MOD_RES (1)..(6): backbone cyclization between the N-alpha-omega-functionalized derivative of X1 and the N-alpha-omega-functionalized derivative of X6
  MOD_RES (4)..(4): D-Trp
  MOD_RES (5)..(5): D-Lys
  MOD_RES (6)..(6): PheN2 building unit
  MOD_RES (6)..(6): AMIDATION
FFFWKF

SEQ ID NO: 16 - protein, 7 aa, Artificial Sequence
  Synthetic peptide
  MOD_RES (1)..(1): PheN2 building unit
  MOD_RES (1)..(6): backbone cyclization between the N-alpha-omega-functionalized derivative of X1 and the N-alpha-omega-functionalized derivative of X6
  MOD_RES (3)..(3): D-2-naphtylalanine
  MOD_RES (6)..(6): GlyC2 building unit
  MOD_RES (7)..(7): AMIDATION
FYXKVGT

SEQ ID NO: 17 - protein, 7 aa, Artificial Sequence
  Synthetic peptide
  MOD_RES (1)..(1): PheN2 building unit
  MOD_RES (1)..(6): backbone cyclization between the N-alpha-omega-functionalized derivative of X1 and the N-alpha-omega-functionalized derivative of X6
  MOD_RES (3)..(3): D-Trp
  MOD_RES (6)..(6): GlyC2 building unit
  MOD_RES (7)..(7): AMIDATION
  MOD_RES (7)..(7): 2-naphtylalanine
FYWKVGX

SEQ ID NO: 18 - protein, 7 aa, Artificial Sequence
  Synthetic peptide
  MOD_RES (1)..(1): PheN2 building unit
  MOD_RES (1)..(7): backbone cyclization between the N-alpha-omega-functionalized derivative of X1 and the N-alpha-omega-functionalized derivative of X7
  MOD_RES (3)..(3): D-Trp
  MOD_RES (7)..(7): GlyC2 building unit
  MOD_RES (7)..(7): AMIDATION
FYWKVVG

SEQ ID NO: 19 - protein, 7 aa, Artificial Sequence
  Synthetic peptide
  MOD_RES (1)..(1): PheN2 building unit
  MOD_RES (1)..(7): backbone cyclization between the N-alpha-omega-functionalized derivative of X1 and the N-alpha-omega-functionalized derivative of X7
  MOD_RES (3)..(3): D-Trp
  MOD_RES (6)..(6): Naphtylalanine
  MOD_RES (7)..(7): GlyC2 building unit
  MOD_RES (7)..(7): AMIDATION
FYWKSXG

SEQ ID NO: 20 - protein, 7 aa, Artificial Sequence
  Synthetic peptide
  MOD_RES (1)..(1): PheN2 building unit
  MOD_RES (1)..(7): backbone cyclization between the N-alpha-omega-functionalized derivative of X1 and the N-alpha-omega-functionalized derivative of X7
  MOD_RES (3)..(3): D-Trp
  MOD_RES (6)..(6): 2-naphtylalanine
  MOD_RES (7)..(7): GlyC2 building unit
  MOD_RES (7)..(7): AMIDATION
FFWKTXG

SEQ ID NO: 21 - protein, 8 aa, Artificial Sequence
  Synthetic peptide
  MOD_RES (1)..(8): backbone cyclization with disulfide bond between the N-alpha-omega-S-functionalized derivative of X8 and the side chain of the X1 Cysteine
  MOD_RES (4)..(4): D-Trp
  MOD_RES (8)..(8): GlyS2 building unit
  MOD_RES (8)..(8): AMIDATION
CFWWKTFG

SEQ ID NO: 22 - protein, 9 aa, Artificial Sequence
  Synthetic peptide
  MOD_RES (1)..(1): D-Phe
  MOD_RES (2)..(9): Backbone cyclization with disulfide bridge between the N-alpha-omega-S-functionalized derivative of X9 and the side chain of the X2 Cys residue
  MOD_RES (5)..(5): D-Trp
  MOD_RES (9)..(9): GlyS2 building unit
  MOD_RES (9)..(9): AMIDATION
FCFWWKTFG

SEQ ID NO: 23 - protein, 8 aa, Artificial Sequence
  Synthetic peptide
  CARBOHYD (1)..(1): Galactose
  MOD_RES (1)..(1): Dbu - 2,4 diaminobutiric acid
  MOD_RES (1)..(8): Backbone cyclization between the N-alpha-omega-functionalized derivative of X8 and the free amino group of X1
  MOD_RES (4)..(4): D-Trp
  MOD_RES (8)..(8): GlyC3 building unit
  MOD_RES (8)..(8): AMIDATION
XFWWKTFG